European Patent Specification EP 4 735 036 B1, published July 22, 2026. Title: IMMUNOTHERAPEUTIC METHODS, COMPOUNDS, AND COMPOSITIONS FOR TREATING OR PREVENTING CELIAC DISEASE. Applicant: DBV TECHNOLOGIES. Application EP. The sequence listing filed with the application follows.

SEQUENCE LISTING (90 sequences)

SEQ ID NO: 1 - protein, 9 aa, synthetic construct
PFPQPZLPY

SEQ ID NO: 2 - protein, 9 aa, synthetic construct
PYPQPZLPY

SEQ ID NO: 3 - protein, 9 aa, synthetic construct
PQPZLPYPQ

SEQ ID NO: 4 - protein, 9 aa, synthetic construct
ZGSFQPSQZ

SEQ ID NO: 5 - protein, 9 aa, synthetic construct
PQQSFPZQZ

SEQ ID NO: 6 - protein, 9 aa, synthetic construct
ZQPZQPFPZ

SEQ ID NO: 7 - protein, 9 aa, synthetic construct
QQPFPZQPQ

SEQ ID NO: 8 - protein, 9 aa, synthetic construct
PFPQPZQPF

SEQ ID NO: 9 - protein, 9 aa, synthetic construct
PQPZQPFPW

SEQ ID NO: 10 - protein, 9 aa, synthetic construct
PQQSFPEQE

SEQ ID NO: 11 - protein, 7 aa, synthetic construct
QPEQPFP

SEQ ID NO: 12 - protein, 9 aa, synthetic construct
EQPEQPFPE

SEQ ID NO: 13 - protein, 9 aa, synthetic construct
ZGSVQPQZL

SEQ ID NO: 14 - protein, 25 aa, synthetic construct
PFPQPZLPYPQPZLPYPQPZLPYPQ

SEQ ID NO: 15 - protein, 31 aa, synthetic construct
QLQPFPQPZLPYPQPZLPYPQPZLPYPQPQP

SEQ ID NO: 16 - protein, 15 aa, synthetic construct
PQPZQPZQPFPZQPQ

SEQ ID NO: 17 - protein, 21 aa, synthetic construct
QQFPQPZQPZQPFPZQPQQQF

SEQ ID NO: 18 - protein, 15 aa, synthetic construct
PSGZGSFQPSQZNPQ

SEQ ID NO: 19 - protein, 21 aa, synthetic construct
QQYPSGZGSFQPSQZNPQAQG

SEQ ID NO: 20 - protein, 17 aa, synthetic construct
PQQPFPQPZQPFPWQPQ

SEQ ID NO: 21 - protein, 23 aa, synthetic construct
PQQPQQPFPQPZQPFPWQPQQPF

SEQ ID NO: 22 - protein, 94 aa, synthetic construct
  VARIANT 54: note = X is P, C or A
QLQPFPQPZLPYPQPZLPYPQPZLPYPQPQPGPRRKKPQPZQPZQPFPZQPQGXRRKKPQQPFPQPZQPFPWQPQGPKKPSGZGSFQPSQZNPQ

SEQ ID NO: 23 - protein, 94 aa, synthetic construct
  VARIANT 54: note = X is P, C or A
QLQPFPQPELPYPQPELPYPQPELPYPQPQPGPRRKKPQPEQPEQPFPEQPQGXRRKKPQQPFPQPEQPFPWQPQGPKKPSGEGSFQPSQENPQ

SEQ ID NO: 24 - protein, 94 aa, synthetic construct
QLQPFPQPELPYPQPELPYPQPELPYPQPQPGPKKRKPQPEQPEQPFPEQPQGPKKRKPQQPFPQPEQPFPWQPQGPKKPSGEGSFQPSQENPQ

SEQ ID NO: 25 - protein, 95 aa, synthetic construct
LQLQPFPQPELPYPQPELPYPQPELPYPQPQPGPKKRKPQPEQPEQPFPEQPQGPKKRKPQQPFPQPEQPFPWQPQGPKKPSGEGSFQPSQENPQ

SEQ ID NO: 26 - protein, 91 aa, synthetic construct
LQLQPFPQPELPYPQPELPYPQPELPYPQPQPGPKKPQPEQPEQPFPEQPQGPKKPQQPFPQPEQPFPWQPQGPKKPSGEGSFQPSQENPQ

SEQ ID NO: 27 - protein, 91 aa, synthetic construct
LQLQPFPQPELPYPQPELPYPQPELPYPQPQPKGKKPQPEQPEQPFPEQPQKGKKPQQPFPQPEQPFPWQPQGPKKPSGEGSFQPSQENPQ

SEQ ID NO: 28 - protein, 11 aa, synthetic construct
PFPQPZQPFPW

SEQ ID NO: 29 - protein, 9 aa, synthetic construct
EGSFQPSQE

SEQ ID NO: 30 - protein, 11 aa, synthetic construct
PFPQPEQPFPW

SEQ ID NO: 31 - protein, 33 aa, synthetic construct
LQLQPFPQPZLPYPQPZLPYPQPZLPYPQPQPF

SEQ ID NO: 32 - protein, 4 aa, synthetic construct
KKKK

SEQ ID NO: 33 - protein, 6 aa, synthetic construct
GPRRKK

SEQ ID NO: 34 - protein, 4 aa, synthetic construct
GPKK

SEQ ID NO: 35 - protein, 6 aa, synthetic construct
GARRKK

SEQ ID NO: 36 - protein, 6 aa, synthetic construct
GCRRKK

SEQ ID NO: 37 - protein, 4 aa, synthetic construct
RVRR

SEQ ID NO: 38 - protein, 4 aa, synthetic construct
GAGA

SEQ ID NO: 39 - protein, 4 aa, synthetic construct
AGAG

SEQ ID NO: 40 - protein, 4 aa, synthetic construct
KGKG

SEQ ID NO: 41 - protein, 5 aa, synthetic construct
GPGPG

SEQ ID NO: 42 - protein, 92 aa, synthetic construct
PQPEQPEQPFPEQPQKGKKLQLQPFPQPELPYPQPELPYPQPELPYPQPQPFKGKKPQQPFPQPEQPFPWQPQKGKKPSGEGSFQPSQENPQ

SEQ ID NO: 43 - protein, 92 aa, synthetic construct
PQQPFPQPEQPFPWQPQKGKKPQPEQPEQPFPEQPQKGKKLQLQPFPQPELPYPQPELPYPQPELPYPQPQPFKGKKPSGEGSFQPSQENPQ

SEQ ID NO: 44 - protein, 90 aa, synthetic construct
QLQPFPQPZLPYPQPZLPYPQPZLPYPQPQPKKKKPQPZQPZQPFPZQPQKKKKPQQPFPQPZQPFPWQPQKKKKPSGZGSFQPSQZNPQ

SEQ ID NO: 45 - protein, 4 aa, synthetic construct
KGKK

SEQ ID NO: 46 - protein, 90 aa, synthetic construct
QLQPFPQPELPYPQPELPYPQPELPYPQPQPKKKKPQPEQPEQPFPEQPQKKKKPQQPFPQPEQPFPWQPQKKKKPSGEGSFQPSQENPQ

SEQ ID NO: 47 - protein, 15 aa, synthetic construct
LQPFPQPELPYPQPQ

SEQ ID NO: 48 - protein, 14 aa, synthetic construct
QPFPQPEQPFPWQP

SEQ ID NO: 49 - protein, 94 aa, synthetic construct
QLQPFPQPELPYPQPELPYPQPELPYPQPQPGPRRKKPQPEQPEQPFPEQPQGCRRKKPQQPFPQPEQPFPWQPQGPKKPSGEGSFQPSQENPQ

SEQ ID NO: 50 - protein, 94 aa, synthetic construct
QLQPFPQPELPYPQPELPYPQPELPYPQPQPGPRRKKPQPEQPEQPFPEQPQGARRKKPQQPFPQPEQPFPWQPQGPKKPSGEGSFQPSQENPQ

SEQ ID NO: 51 - protein, 9 aa, synthetic construct
PFPQPELPY

SEQ ID NO: 52 - protein, 9 aa, synthetic construct
PFPQPQLPY

SEQ ID NO: 53 - protein, 9 aa, synthetic construct
PYPQPELPY

SEQ ID NO: 54 - protein, 9 aa, synthetic construct
PYPQPQLPY

SEQ ID NO: 55 - protein, 9 aa, synthetic construct
PQPELPYPQ

SEQ ID NO: 56 - protein, 9 aa, synthetic construct
PQPQLPYPQ

SEQ ID NO: 57 - protein, 9 aa, synthetic construct
EGSFQPSQE

SEQ ID NO: 58 - protein, 9 aa, synthetic construct
QGSFQPSQQ

SEQ ID NO: 59 - protein, 9 aa, synthetic construct
EGSFQPSQQ

SEQ ID NO: 60 - protein, 9 aa, synthetic construct
QGSFQPSQE

SEQ ID NO: 61 - protein, 9 aa, synthetic construct
PQQSFPEQE

SEQ ID NO: 62 - protein, 9 aa, synthetic construct
PQQSFPQQQ

SEQ ID NO: 63 - protein, 9 aa, synthetic construct
PQQSFPEQQ

SEQ ID NO: 64 - protein, 9 aa, synthetic construct
PQQSFPQQE

SEQ ID NO: 65 - protein, 9 aa, synthetic construct
EQPEQPFPE

SEQ ID NO: 66 - protein, 9 aa, synthetic construct
QQPQQPFPQ

SEQ ID NO: 67 - protein, 9 aa, synthetic construct
EQPEQPFPQ

SEQ ID NO: 68 - protein, 9 aa, synthetic construct
EQPQQPFPE

SEQ ID NO: 69 - protein, 9 aa, synthetic construct
QQPQQPFPE

SEQ ID NO: 70 - protein, 9 aa, synthetic construct
QQPEQPFPQ

SEQ ID NO: 71 - protein, 9 aa, synthetic construct
EQPQQPFPQ

SEQ ID NO: 72 - protein, 9 aa, synthetic construct
QQPEQPFPE

SEQ ID NO: 73 - protein, 9 aa, synthetic construct
QQPFPEQPQ

SEQ ID NO: 74 - protein, 9 aa, synthetic construct
QQPFPQQPQ

SEQ ID NO: 75 - protein, 9 aa, synthetic construct
PFPQPEQPF

SEQ ID NO: 76 - protein, 9 aa, synthetic construct
PFPQPQQPF

SEQ ID NO: 77 - protein, 9 aa, synthetic construct
PQPEQPFPW

SEQ ID NO: 78 - protein, 9 aa, synthetic construct
PQPQQPFPW

SEQ ID NO: 79 - protein, 9 aa, synthetic construct
EGSVQPQEL

SEQ ID NO: 80 - protein, 9 aa, synthetic construct
QGSVQPQQL

SEQ ID NO: 81 - protein, 9 aa, synthetic construct
EGSVQPQQL

SEQ ID NO: 82 - protein, 9 aa, synthetic construct
QGSVQPQEL

SEQ ID NO: 83 - protein, 31 aa, synthetic construct
QLQPFPQPELPYPQPELPYPQPELPYPQPQP

SEQ ID NO: 84 - protein, 15 aa, synthetic construct
PQPEQPEQPFPEQPQ

SEQ ID NO: 85 - protein, 17 aa, synthetic construct
PQQPFPQPEQPFPWQPQ

SEQ ID NO: 86 - protein, 15 aa, synthetic construct
PSGEGSFQPSQENPQ

SEQ ID NO: 87 - protein, 7 aa, synthetic construct
PFPLPQP

SEQ ID NO: 88 - protein, 7 aa, synthetic construct
PQYQPEQ

SEQ ID NO: 89 - protein, 7 aa, synthetic construct
PFEPQPL

SEQ ID NO: 90 - protein, 7 aa, synthetic construct
PQSYPEQ